European Patent Application EP 4 279 587 A1, published November 22, 2023. Title: Engineered microorganisms expressing acetoacetyl-CoA reductase variants and methods for increasing proportion of 3-hydroxyhexanoic acid in PHA. Applicant: Shenzhen Bluepha Biosciences Co., Ltd. The sequence listing filed with the application follows.

SEQUENCE LISTING (36 sequences)

SEQ ID NO: 1 - DNA, 741 bp, Artificial Sequence
  Laboratory synthesis
atgcagagccgcgtggccctggtgaccggcggcaccggcggcatcggcacctcgatcatccagcgcctggcccagaccggccaccgcgtggccaccaactaccgcgacgaggaccgcgcgcgcgcctggcaggagaagatgcgcgcggccggcgtggaggtggccctggccccgggcgacgtgtcgagcccggagcaggcccaggccctggtggagcagatccagcgcgacctgggcccgatcgaggtgctggtgaacaacgccggcatcacccgcgactcgaccttccaccgcatgaccccgctgcagtggaacgaggtgatcggcaccaacctgaacagctgcttcaacgtgacccgcccggtgatcgagggcatgcgcgagcgcaagtggggccgcatcgtgcagatctcgagcatcaacggcctgaagggccagtacggccaggccaactacgcggccgccaaggcgggcatgcacggcttcaccatcagcctggcccgcgagaacgcccgcttcggcgtgaccgtgaacaccgtgtcgccgggctacgtggccaccgacatggtgatgagcgtgccggaggaagtgcgcgcgaagatcgtggcggagatcccgaccggccgcctgggcaccccgaacgagatcgcgtacgccgtgtcgttcctggtggcggaggaagccgcctggatcaccggcagcaacctggacatcaacggtggccaccacatgggctggtaa

SEQ ID NO: 2 - DNA, 741 bp, Artificial Sequence
  Laboratory synthesis
atgcagaagctggccctgatcaccggcagcaagggcggcatcggctcggccatcaccgagaagctggtgcaggacggcttccgcatcatcgcgacctacttcaccggcaactacgagtgcgccaaggagtggttcgacgagaagggcttcagcgaggaccaggtgaccctgttcgagctggacgtgaccgacgcggacagctgccgcgagcgcctgaccaagctgctggagaacgagggcaccgtggacgtgctggtgaacaacgcgggcatcacccgcgactgcaccttcaagcgcatgaccgccgagcagtggaacgacgtgatcaacaccaacctgaacagcgtgttcaacgtgacccagccgctgttcgcggccatgtgcgagaagggcggcggccgcatcatcaacatctcgagcgtgaacggcctgaagggccagttcggccagaccaactactcggccgcgaaggcgggcatgatcggcttcagcaaggccctggccttcgagggcgcccgcagcggcgtgaccgtgaacgtggtggccccgggctacaccggcaccccgatggtgcaggccatccgccaggacgtgctggacagcatcatcgaaaccgtgccgatgaagcgcctggccaccccggaggagatcgccagcgccgtggcctacctggcctcggacgccggcgcctacatcaccggcgaaaccctgagcgtgaacggcggcctgtacatgcagtaa

SEQ ID NO: 3 - DNA, 816 bp, Artificial Sequence
  Laboratory synthesis
atgaccaccgccgcggccgagaagcgcgcggccaccaactcgggctcggagccggtgcgcgaggccgtgccgccgctgaagcagcgcatcgccttcgtgtcgggcggcatgggcggcatcggcagcgcggtgtgccgtcgcctggtgcgcaacggcgcccgcgtggtggcgggctgcctgccgggctacgagaagaaggacgagtggatcgccaagatgcgcggcgagggcctgcaggtgcacgccgccgagggcgacgtggacgactacgagtcgtgcgcggacatgttctaccagatcggcagcgtgatcggcccggtggacatcctggtgaacaacgccggcatcacccgcgacggcatgttcaagcgcatgagcccggccgactggtacgccgtgatcaacaccaacctgaacagcgtgttcaacgtgacccgccaggtgatcgagggcatgatggagcgcggctggggccgcatcatcaacatctcgagcgtgaacgcgctgaagggccagttcggccagaccaactacagcgccgccaaggcgggcatgcacggcttcagcaaggcgctggcccaggaagtggtgaagaagggcgtgaccgtgaacaccgtgtcgccgggctacgtggaaaccgacatggtgcgcgccatgaagccggaggtgctgcagagcatcgtggagcagatcccgatgggccgcttcgcccagccggaggagatcgccagcctggtggcctacctggcctcggaggaagccggctacatcaccggcgccaacatctcgatcaacggcggcctgcacatggtgtaa

SEQ ID NO: 4 - DNA, 747 bp, Artificial Sequence
  Laboratory synthesis
atggcgaaccaggccccggtggcctgggtgaccggcggcaccggcggcatcggcaccgccatctgccgctcgctggcggacgccggctacctggtggtggccggctaccacaacccggagaaggccaagacctggctggccagccagcaggccgacggctacaacaacatcgccctgagcggcgtggacctggcggaccaccaggcctgcctgcagggcgcccagcagatccaggagcagcacggcccgatctcggtgctggtgaactgcgcgggcatcacccgcgacggcaccatgaagaagatgagctacgagcagtggtacgaggtgatcgacaccaacctgaactcggtgttcaacacctgccgcagcgtgatcgagatgatgctggagaacggctacggccgcatcatcaacatctcgagcatcaacggccgcaagggccagttcggccaggccaactacgcggccgccaaggccggcatgcacggcctgaccatgtcgctggcccaggaaaccgcgaccaagggcatcaccgtgaacaccgtgagcccgggctacatcgccaccgacatgatcatgaacatcccggagaaggtgcgcgaggccatccgcgaaaccatcccggtgaagcgctacggcaccccggaggagatcggccgcctggtgaccttcatcgccgacaaggagagcggcttcatcaccggcgcgaacttcgacatcaacggtggccagttcatgggctaa

SEQ ID NO: 5 - DNA, 741 bp, Artificial Sequence
  Laboratory synthesis
atgtcgcgcgtggccctggtgaccggcggcatgggcggcctgggcgaggcgatctgcatcaagatggcggccctgggctaccaggtggtgaccacctactcgccgggcaacaagacctggaaggagtggctggacagcatgaacaagatgggcttcggcttccgcgcctacccgtgcgacgtggccgactacgacagcgccaccgcctgcgtggccctgatcgtgaaggaagtgggcccggtggacgtgctggtgaacaacgcgggcatcacccgcgacatgaccttcaagaagatggacaagatcaactgggacgccgtggtggcgaccaacctggacagcaccttcaacatgaccaagcaggtgtgcgacggcatgctggagcgcggctggggccgcatcgtgaacatctcgtcggtgaacggccagaagggcgccttcggccagaccaactacagcgcggccaaggccggcatgcacggcttcaccaaggccctggccctggaggtggcccgcaagggcgtgaccgtgaacaccatcagcccgggctacatcggcaccaagatggtgatggcgatcccgtcggacgtgctggagagcaagatcatcccgcagatcccgatgggccgcctgggcaagccggaggaagtggcgggcctggtggcctacctggccagcgacgaggcggcgttcctgaccggcgccaacatcgcgatcaacggtggccagcacatgagctaa

SEQ ID NO: 6 - DNA, 744 bp, Artificial Sequence
  Laboratory synthesis
atgacccagcgcatcgccatcgtgaccggcgccaacggcggcctgggcgagagcatgtgcaaggccctggccgagcagggccgcaaggtggtgggcaccttcgtgccgggccacgacgcggccgcggccagctggcaggaagagatgaagcagcagggcttcgacatcaccatgaaggccgtggacgtgtcggacttcaacgactgcaagcgcctgctggaggagatcgagtcgagcgagggcagcgtggacatcctggtgaacaacgcgggcatcacccgcgacgcgccgctgaagaagatgcagccggagcagtggcaggcggtgatcggcaccaacctgaactcgatgttcaacatgagccagccgatcttcgaggccatgtgcaaccgcggctggggccgcatcgtgaacatctcgagcctgaacggcgagaagggccagttcggccaggccaactacagcgcggccaaggcgggcatctacggcttcaccaaggccatcgcgcaggaaggcgccaagaagggcgtgaccgtgaactcggtgagcccgggctacatcgacaccccgatggtgcgccaggtgccggagaacgtgctgaacagcatcgtgggcggcatcccggtgggccgcctgggccagccggaggagatcgcccgcgcggtgtcgttcctgaccgcggacgacgccggcttcatcaccggcaccaacatcagcgtgaacggtggccagtacatggcgtaa

SEQ ID NO: 7 - DNA, 741 bp, Artificial Sequence
  Laboratory synthesis
atgtcgcgcgtggccctggtgaccggcggcatgggcggcctgggcgaggcgatctgcatcaagctggccgcgctgggctacaaggtggtgaccacccacagcccgggcaacaccaaggcggccgagtggctgctgaccatgaacaacatgggctacggcttcaaggcctacccgtgcgacgtgagcgacttcgactcgagcaaggcgtgcgtggaaaccgtgacccgcgaagtgggcccggtggacgtgctggtgaacaacgccggcatcacccgcgacatgaccttcaagaagatgaccaaggccgactgggacgcggtgatcggcaccaacctggactcggtgttcaacatgaccaagcaggtgatggacggcatggtggagcgtcgctggggccgcgtgatcaacgtgtcgtcggtgaacggccagaagggcgccttcggccagaccaactactcggcggccaaggccggcatgcacggcttcaccaaggccctggccctggaggtggcccgcaacggcgtgaccgtgaacaccatctcgccgggctacatcggcaccaagatggtgatggccatcccgcaggagatcctggacagcaagatcctgccgcagatcccgctggcccgcctgggcaagccggaggagatcgcgggcctggtggcctacctgagctcggaggaagccgccttcgtgaccggcgcgaacatcagcatcaacggtggccagcacatgttctaa

SEQ ID NO: 8 - DNA, 2887 bp, Artificial Sequence
  Laboratory synthesis
cgggcgtgcccatgatgtagagcaccagcgccaccggcgccatgccatacatcaggaaggtggcaacgcctgccaccacgttgtgctcggtgatcgccatcatcagcgccacgtagagccagccaatggccacgatgtacatcaaaaattcatccttctcgcctatgctctggggcctcggcagatgcgagcgctgcataccgtccggtaggtcgggaagcgtgcagtgccgaggcggattcccgcattgacagcgcgtgcgttgcaaggcaacaatggactcaaatgtctcggaatcgctgacgattcccaggtttctccggcaagcatagcgcatggcgtctccatgcgagaatgtcgcgcttgccggataaaaggggagccgctatcggaatggacgcaagccacggccgcagcaggtgcggtcgagggcttccagccagttccagggcagatgtgccggcagaccctcccgctttgggggaggcgcaagccgggtccattcggatagcatctccccatgcaaagtgccggccagggcaatgcccggagccggttcgaatagtgacggcagagagacaatcaaatcatgagccaaccatcttatggcccgctgttcgaggccctggcccactacaatgacaagctgctggccatggccaaggcccagacagagcgcaccgcccaggcgctgctgcagaccaatctggacgatctgggccaggtgctggagcagggcagccagcaaccctggcagctgatccaggcccagatgaactggtggcaggatcagctcaagctgatgcagcacaccctgctcaaaagcgcaggccagccgagcgagccggtgatcaccccggagcgcagcgatcgccgcttcaaggccgaggcctggagcgaacaacccatctatgactacctcaagcagtcctacctgctcaccgccaggcacctgctggcctcggtggatgccctggagggcgtcccccagaagagccgggagcggctgcgtttcttcacccgccagtacgtctctgccatggcccccagcaacttcctggccaccaaccccgagctgctcaagctgaccctggagtccggcggccagaacctggtgcgcggactggccctcttggccgaggatctggagcgcagcgccgatcagctcaacatccgcctgaccgacgaatccgccttcgagctcgggcgggatctggccctgaccccgggccgggtggtgcagcgcaccgagctctatgagctcattcagtacagcccgactaccgagacggtgggcaagacacctgtgctgatagtgccgcccttcatcaacaagtactacatcatggacatgcggccccagaactccctggtcgcctggctggtcgcccagggccagacggtattcatgatctcctggcgcaacccgggcgtggcccaggcccaaatcgatctcgacgactacgtggtggatggcgtcatcgccgccctggacggcgtggaggcggccaccggcgagcgggaggtgcacggcatcggctactgcatcggcggcaccgccctgtcgctcgccatgggctggctggcggcgcggcgccagaagcagcgggtgcgcaccgccaccctgttcactaccctgctggacttctcccagcccggggagcttggcatcttcatccacgagcccatcatagcggcgctcgaggcgcaaaatgaggccaagggcatcatggacgggcgccagctggcggtcagcttcagcctgctgcgggagaacagcctctactggaactactacatcgacagctacctcaagggtcagagcccggtggccttcgatctgctgcactggaacagcgacagcaccaatgtggcgggcaagacccacaacagcctgctgcgccgtctctacctggagaaccagctggtgaagggggagctcaagatccgcaacacccgcatcgatctcggcaaggtgaagacccctgtgctgctggtgtcggcggtggacgatcacatcgccctctggcagggcacctggcagggcatgaagctgtttggcggggagcagcgcttcctcctggcggagtccggccacatcgccggcatcatcaacccgccggccgccaacaagtacggcttctggcacaacggggccgaggccgagagcccggagagctggctggcaggggcgacgcaccagggcggctcctggtggcccgagatgatgggctttatccagaaccgtgacgaagggtcagagcccgtccccgcgcgggtcccggaggaagggctggcccccgcccccggccactatgtcaaggtgcggctcaaccccgtgtttgcctgcccaacagaggaggacgccgcatgacgcttgcatgagtgccggcgtgcgtcatgcacggcgccggcaggcctgcaggttccctcccgtttccattgaaaggactacacaatgactgacgttgtcatcgtatccgccgcccgcaccgcggtcggcaagtttggcggctcgctggccaagatcccggcaccggaactgggtgccgtggtcatcaaggccgcgctggagcgcgccggcgtcaagccggagcaggtgagcgaagtcatcatgggccaggtgctgaccgccggttcgggccagaaccccgcacgccaggccgcgatcaaggccggcctgccggcgatggtgccggccatgaccatcaacaaggtgtgcggctcgggcctgaaggccgtgatgctggccgccaacgcgatcatggcgggcgacgccgagatcgtggtggccggcggccaggaaaacatgagcgccgccccgcacgtgctgccgggctcgcgcgatggtttccgcatgggcgatgccaagctggtcgacaccatg

SEQ ID NO: 9 - protein, 246 aa, Artificial Sequence
  Laboratory synthesis
MQSRVALVTGGTGGIGTSIIQRLAQTGHRVATNYRDEDRARAWQEKMRAAGVEVALAPGDVSSPEQAQALVEQIQRDLGPIEVLVNNAGITRDSTFHRMTPLQWNEVIGTNLNSCFNVTRPVIEGMRERKWGRIVQISSINGLKGQYGQANYAAAKAGMHGFTISLARENARFGVTVNTVSPGYVATDMVMSVPEEVRAKIVAEIPTGRLGTPNEIAYAVSFLVAEEAAWITGSNLDINGGHHMGW

SEQ ID NO: 10 - protein, 246 aa, Artificial Sequence
  Laboratory synthesis
MQKLALITGSKGGIGSAITEKLVQDGFRIIATYFTGNYECAKEWFDEKGFSEDQVTLFELDVTDADSCRERLTKLLENEGTVDVLVNNAGITRDCTFKRMTAEQWNDVINTNLNSVFNVTQPLFAAMCEKGGGRIINISSVNGLKGQFGQTNYSAAKAGMIGFSKALAFEGARSGVTVNVVAPGYTGTPMVQAIRQDVLDSIIETVPMKRLATPEEIASAVAYLASDAGAYITGETLSVNGGLYMQ

SEQ ID NO: 11 - protein, 271 aa, Artificial Sequence
  Laboratory synthesis
MTTAAAEKRAATNSGSEPVREAVPPLKQRIAFVSGGMGGIGSAVCRRLVRNGARVVAGCLPGYEKKDEWIAKMRGEGLQVHAAEGDVDDYESCADMFYQIGSVIGPVDILVNNAGITRDGMFKRMSPADWYAVINTNLNSVFNVTRQVIEGMMERGWGRIINISSVNALKGQFGQTNYSAAKAGMHGFSKALAQEVVKKGVTVNTVSPGYVETDMVRAMKPEVLQSIVEQIPMGRFAQPEEIASLVAYLASEEAGYITGANISINGGLHMV

SEQ ID NO: 12 - protein, 248 aa, Artificial Sequence
  Laboratory synthesis
MANQAPVAWVTGGTGGIGTAICRSLADAGYLVVAGYHNPEKAKTWLASQQADGYNNIALSGVDLADHQACLQGAQQIQEQHGPISVLVNCAGITRDGTMKKMSYEQWYEVIDTNLNSVFNTCRSVIEMMLENGYGRIINISSINGRKGQFGQANYAAAKAGMHGLTMSLAQETATKGITVNTVSPGYIATDMIMNIPEKVREAIRETIPVKRYGTPEEIGRLVTFIADKESGFITGANFDINGGQFMG

SEQ ID NO: 13 - protein, 246 aa, Artificial Sequence
  Laboratory synthesis
MSRVALVTGGMGGLGEAICIKMAALGYQVVTTYSPGNKTWKEWLDSMNKMGFGFRAYPCDVADYDSATACVALIVKEVGPVDVLVNNAGITRDMTFKKMDKINWDAVVATNLDSTFNMTKQVCDGMLERGWGRIVNISSVNGQKGAFGQTNYSAAKAGMHGFTKALALEVARKGVTVNTISPGYIGTKMVMAIPSDVLESKIIPQIPMGRLGKPEEVAGLVAYLASDEAAFLTGANIAINGGQHMS

SEQ ID NO: 14 - protein, 247 aa, Artificial Sequence
  Laboratory synthesis
MTQRIAIVTGANGGLGESMCKALAEQGRKVVGTFVPGHDAAAASWQEEMKQQGFDITMKAVDVSDFNDCKRLLEEIESSEGSVDILVNNAGITRDAPLKKMQPEQWQAVIGTNLNSMFNMSQPIFEAMCNRGWGRIVNISSLNGEKGQFGQANYSAAKAGIYGFTKAIAQEGAKKGVTVNSVSPGYIDTPMVRQVPENVLNSIVGGIPVGRLGQPEEIARAVSFLTADDAGFITGTNISVNGGQYMA

SEQ ID NO: 15 - protein, 246 aa, Artificial Sequence
  Laboratory synthesis
MSQKIALVTGAMGGLGTAICQSLARDGMKVVANCLPGFDQKEGWLAAQRDLGFNFIAAEGDVSDYDSCAAMVARIEAEVGPVDVLVNNAGITRDKFFPKMQKAQWDAVINTNLNSLFNVTHHVSAKMAERGWGRIISISSVNGVKGQAGQTNYSAAKAGVLGFTKALAAELATKGVTVNAVAPGYVGTEMVMAIRDDIRQGIIDTIPMGRLGRPDEIGDLCAYLASDKAAYITGATININGGLHMC

SEQ ID NO: 16 - protein, 593 aa, Artificial Sequence
  Laboratory synthesis
MSQPSYGPLFEALAHYNDKLLAMAKAQTERTAQALLQTNLDDLGQVLEQGSQQPWQLIQAQMNWWQDQLKLMQHTLLKSAGQPSEPVITPERSDRRFKAEAWSEQPIYDYLKQSYLLTARHLLASVDALEGVPQKSRERLRFFTRQYVSAMAPSNFLATNPELLKLTLESGGQNLVRGLALLAEDLERSADQLNIRLTDESAFELGRDLALTPGRVVQRTELYELIQYSPTTETVGKTPVLIVPPFINKYYIMDMRPQNSLVAWLVAQGQTVFMISWRNPGVAQAQIDLDDYVVDGVIAALDGVEAATGEREVHGIGYCIGGTALSLAMGWLAARRQKQRVRTATLFTTLLDFSQPGELGIFIHEPIIAALEAQNEAKGIMDGRQLAVSFSLLRENSLYWNYYIDSYLKGQSPVAFDLLHWNSDSTNVAGKTHNSLLRRLYLENQLVKGELKIRNTRIDLGKVKTPVLLVSAVDDHIALWQGTWQGMKLFGGEQRFLLAESGHIAGIINPPAANKYGFWHNGAEAESPESWLAGATHQGGSWWPEMMGFIQNRDEGSEPVPARVPEEGLAPAPGHYVKVRLNPVFACPTEEDA

SEQ ID NO: 17 - DNA, 169 bp, Artificial Sequence
  Laboratory synthesis
atgcctccacaccgctcgtcacatcctgttgcgttcactggaatcccagtatctaatttgacctgcgagcaagctgtcaccggatgtgctttccggtctgatgagtccgtgaggacgaaacagcctctacaaataattttgtttaactgactgaattcatgggacaagc

SEQ ID NO: 18 - DNA, 20 bp, Artificial Sequence
  Laboratory synthesis
gcagacttggccgggtacca

SEQ ID NO: 19 - DNA, 19 bp, Artificial Sequence
  Laboratory synthesis
caccgctcgtcacatcctg

SEQ ID NO: 20 - DNA, 40 bp, Artificial Sequence
  Laboratory synthesis
tggtacccggccaagtctgcgggcgtgcccatgatgtaga

SEQ ID NO: 21 - DNA, 42 bp, Artificial Sequence
  Laboratory synthesis
tgagacccaaggtctccatgatttgattgtctctctgccgtc

SEQ ID NO: 22 - DNA, 38 bp, Artificial Sequence
  Laboratory synthesis
ggagaccttgggtctcagtgacgcttgcatgagtgccg

SEQ ID NO: 23 - DNA, 39 bp, Artificial Sequence
  Laboratory synthesis
caggatgtgacgagcggtgcatggtgtcgaccagcttgg

SEQ ID NO: 24 - DNA, 11 bp, Artificial Sequence
  Laboratory synthesis
gtgaagagacc

SEQ ID NO: 25 - DNA, 21 bp, Artificial Sequence
  Laboratory synthesis
tggtctggctggcggactgag

SEQ ID NO: 26 - DNA, 21 bp, Artificial Sequence
  Laboratory synthesis
ggcgaactcatcctgcgcctc

SEQ ID NO: 27 - DNA, 24 bp, Artificial Sequence
  Laboratory synthesis
catgatttgattgtctctctgccg

SEQ ID NO: 28 - DNA, 20 bp, Artificial Sequence
  Laboratory synthesis
gtgacgcttgcatgagtgcc

SEQ ID NO: 29 - DNA, 39 bp, Artificial Sequence
  Laboratory synthesis
agagagacaatcaaatcatgactcagcgcattgcgtatg

SEQ ID NO: 30 - DNA, 40 bp, Artificial Sequence
  Laboratory synthesis
ggcactcatgcaagcgtcactcagcccatatgcaggccgc

SEQ ID NO: 31 - DNA, 37 bp, Artificial Sequence
  Laboratory synthesis
tggtacccggccaagtctgttcgacggcgtcttcgtt

SEQ ID NO: 32 - DNA, 38 bp, Artificial Sequence
  Laboratory synthesis
cgagcggtgtggaggcatctattcagtcagggatgcct

SEQ ID NO: 33 - DNA, 62 bp, Artificial Sequence
  Laboratory synthesis
ctacaaataattttgtttaactgactgaattcatgggacaagcatgaagacctacgagaaca

SEQ ID NO: 34 - DNA, 41 bp, Artificial Sequence
  Laboratory synthesis
cttgaagacgaaagggcctcgtggcgccttatggaaatcag

SEQ ID NO: 35 - DNA, 18 bp, Artificial Sequence
  Laboratory synthesis
atgcctccacaccgctcg

SEQ ID NO: 36 - DNA, 26 bp, Artificial Sequence
  Laboratory synthesis
ttaaacaaaattatttgtagaggctg